European Patent Specification EP 3 510 172 B1, published November 29, 2023. Title: METHODS OF DETECTING LENTIVIRUS. Applicant: St Vincent's Hospital Sydney Limited. Application EP 17847818.6. The sequence listing filed with the application follows.

SEQUENCE LISTING (53 sequences)

SEQ ID NO: 1 - DNA, 95 bp, Human immunodeficiency virus type 1
gtctctctggttagaccagatctgagcctgggagctctctggctaactagggaacccactgcttaagcctcaataaagcttgccttgagtgcttc

SEQ ID NO: 2 - DNA, 124 bp, Human immunodeficiency virus type 2
ttgagccctgggaggttctctccagcactagcaggtagagcctgggtgttccctgctagactctcaccagcacttggccggtgctgggcagacggccccacgcttgcttgcttaaaaacctcct

SEQ ID NO: 3 - DNA, 17 bp, Human immunodeficiency virus type 1
taagcagtgggttccct

SEQ ID NO: 4 - DNA, 17 bp, Artificial Sequence
  Sequence of the HIV-1 R region probe oligo
agggaacccactgctta

SEQ ID NO: 5 - DNA, 17 bp, Artificial Sequence
  Sequence of the HIV-1 R region probe oligo with reporter and quencher
  misc_feature (1)..(1): Adenine is attached with X wherein X is a reporter molecule
  misc_feature (17)..(17): Adenine is attached with Z wherein  Z is a quencher molecule.
agggaacccactgctta

SEQ ID NO: 6 - DNA, 17 bp, Artificial Sequence
  Sequence of the HIV-1 R region probe oligo with locked nucleic acids
  misc_feature (1)..(1): Adenine is attached with FAM (carboxyfluorescein)
  modified_base (3)..(3): Locked nucleic acid guanine
  modified_base (5)..(5): Locked nucleic acid adenine
  modified_base (7)..(7): Locked nucleic acid cytosine
  modified_base (11)..(11): Locked nucleic acid cytosine
  modified_base (13)..(13): Locked nucleic acid guanine
  misc_feature (17)..(17): Adenine is attached with BHQ-1
agggaacccactgctta

SEQ ID NO: 7 - DNA, 18 bp, Human immunodeficiency virus type 1
gagcctgggagctctctg

SEQ ID NO: 8 - DNA, 18 bp, Human immunodeficiency virus type 1
cagagagctcccaggctc

SEQ ID NO: 9 - DNA, 24 bp, Artificial Sequence
  HIV-1 reverse R region primer
actcaaggcaagctttattgaggc

SEQ ID NO: 10 - DNA, 24 bp, Human immunodeficiency virus type 1
gcctcaataaagcttgccttgagt

SEQ ID NO: 11 - DNA, 25 bp, Human immunodeficiency virus type 2
gcctgggtgttccctgctagactct

SEQ ID NO: 12 - DNA, 25 bp, Artificial Sequence
  Sequence of the HIV-2 R region probe oligo
agagtctagcagggaacacccaggc

SEQ ID NO: 13 - DNA, 25 bp, Artificial Sequence
  Sequence of the HIV-2 R region probe oligo with reporter and quencher
  misc_feature (1)..(1): Adenine is attached with X wherein  X is a reporter molecule
  misc_feature (25)..(25): Cytosine is attached with Z wherein Z is a quencher molecule
agagtctagcagggaacacccaggc

SEQ ID NO: 14 - DNA, 18 bp, Artificial Sequence
  HIV-2 forward R region primer
gagccctgagaggttctc

SEQ ID NO: 15 - DNA, 18 bp, Human immunodeficiency virus type 2
gagaacctcccagggctc

SEQ ID NO: 16 - DNA, 23 bp, Artificial Sequence
  HIV-2 reverse R region primer
ggtctttaagcaagcaagcgtgg

SEQ ID NO: 17 - DNA, 27 bp, Artificial Sequence
  GAPDH probe oligo
  misc_feature (1)..(1): Adenine is attached with FAM (carboxyfluorescein)
  misc_feature (27)..(27): Thymine is attached with quencher molecule BHQ-1
aaggtcggagtcaacggatttggtcgt

SEQ ID NO: 18 - DNA, 23 bp, Artificial Sequence
  GAPDH forward primer
ggcaacaatatccactttaccag

SEQ ID NO: 19 - DNA, 20 bp, Artificial Sequence
  GAPDH reverse primer
tcgacagtcagccgcatctt

SEQ ID NO: 20 - DNA, 25 bp, Artificial Sequence
  B-actin probe oligo
  misc_feature (1)..(1): Adenine is attached with FAM (carboxyfluorescein)
  misc_feature (25)..(25): Guanine is attached with quencher molecule BHQ-1
atgccctcccccatgccatcctgcg

SEQ ID NO: 21 - DNA, 25 bp, Artificial Sequence
  B-actin forward primer
tcacccacactgtgcccatctacga

SEQ ID NO: 22 - DNA, 25 bp, Artificial Sequence
  B-actin reverse primer
cagcggaaccgctcattgccaatgg

SEQ ID NO: 23 - DNA, 24 bp, Artificial Sequence
  3' LTR forward primer
ccaaagaagacaagatatccttga

SEQ ID NO: 24 - DNA, 18 bp, Artificial Sequence
  3' LTR reverse primer
ttgaggcttaagcagtgg

SEQ ID NO: 25 - DNA, 29 bp, Artificial Sequence
  3' LTR probe oligo
  misc_feature (1)..(1): Thymine is attached with FAM (carboxyfluorescein)
  misc_feature (29)..(29): Cytosine is attached with quencher molecule BHQ-1
ttagaccagatctgagcctgggagctctc

SEQ ID NO: 26 - DNA, 30 bp, Artificial Sequence
  gag forward primer
agtggggggacatcaagcagccatgcaaat

SEQ ID NO: 27 - DNA, 28 bp, Artificial Sequence
  gag reverse primer
tactagtagttcctgctatgtcacttcc

SEQ ID NO: 28 - DNA, 17 bp, Artificial Sequence
  gag probe oligo
  misc_feature (1)..(1): Adenine is attached with FAM (carboxyfluorescein)
  modified_base (3)..(3): locked nucleic acid cytosine
  modified_base (4)..(4): locked nucleic acid adenine
  modified_base (7)..(7): locked nucleic acid guanine
  modified_base (13)..(13): locked nucleic acid guanine
  modified_base (16)..(16): locked nucleic acid guanine
  misc_feature (17)..(17): Cytosine is attached with quencher molecule BHQ-1
atcaatgaggaagctgc

SEQ ID NO: 29 - DNA, 18 bp, Artificial Sequence
  HIV-1 forward R region primer (HIV-1 For 2)
  misc_feature (6)..(6): T or C
  misc_feature (15)..(15): T or C
gagccngggagctcnctg

SEQ ID NO: 30 - DNA, 22 bp, Artificial Sequence
  HIV-1 reverse R region primer (HIV-1 Rev 2)
actcaaggcaagctttattgag

SEQ ID NO: 31 - DNA, 18 bp, Artificial Sequence
  HIV-2 forward R region primer (HIV-2 For 1)
  misc_feature (9)..(9): G or A
gagccctgngaggttctc

SEQ ID NO: 32 - DNA, 23 bp, Artificial Sequence
  HIV-2 reverse R region primer (HIV-2 Rev 1)
  misc_feature (4)..(4): T or C
ggtntttaagcaagcaagcgtgg

SEQ ID NO: 33 - DNA, 18 bp, Artificial Sequence
  HIV-2 forward R region primer (HIV-2 For 2)
  misc_feature (9)..(9): G or A
gagccctgngaggttctc

SEQ ID NO: 34 - DNA, 18 bp, Artificial Sequence
  HIV-2 reverse R region primer (HIV-2 Rev 2)
agggaacacccaggctct

SEQ ID NO: 35 - DNA, 19 bp, Artificial Sequence
  HIV-2 forward R region primer (HIV 2 For 3)
ttgagccctgggaggttct

SEQ ID NO: 36 - DNA, 18 bp, Artificial Sequence
  HIV-2 reverse R region primer (HIV-2 Rev 3)
ggaacacccaggctctac

SEQ ID NO: 37 - DNA, 14 bp, Artificial Sequence
  Sequence of the HIV-2 R region probe oligo (HIV-2 Pro 2)
ctgctagtgctgga

SEQ ID NO: 38 - DNA, 14 bp, Artificial Sequence
  Sequence of the HIV-2 R region probe oligo (HIV-2 Pro 2) with reporter and quencher
  misc_feature (1)..(1): Cytosine is attached with X wherein X is a reporter molecule
  misc_feature (14)..(14): Adenine is attached with Z wherein Z is a quencher molecule
ctgctagtgctgga

SEQ ID NO: 39 - DNA, 14 bp, Artificial Sequence
  Sequence of the HIV-2 R region probe oligo (HIV-2 Pro 2) with FAM and BHQ-1
  misc_feature (1)..(1): Cytosine is attached with FAM (carboxyfluorescein)
  misc_feature (14)..(14): Adenine is attached with quencher molecule BHQ-1
ctgctagtgctgga

SEQ ID NO: 40 - DNA, 14 bp, Artificial Sequence
  Sequence of the HIV-2 R region probe oligo (HIV-2 Pro 2) with locked nucleic acids, FAM and BHQ-1
  misc_feature (1)..(1): Cytosine is attached with FAM (carboxyfluorescein)
  modified_base (2)..(2): locked nucleic acid thymine
  modified_base (4)..(4): locked nucleic acid cytosine
  modified_base (6)..(6): locked nucleic acid adenine
  modified_base (8)..(8): locked nucleic acid thymine
  modified_base (9)..(9): locked nucleic acid guanine
  modified_base (13)..(13): locked nucleic acid guanine
  misc_feature (14)..(14): Adenine is attached with quencher molecule BHQ-1
ctgctagtgctgga

SEQ ID NO: 41 - DNA, 14 bp, Artificial Sequence
  Sequence of the HIV-2 R region probe oligo (HIV-2 Pro 3)
tccagcactagcag

SEQ ID NO: 42 - DNA, 14 bp, Artificial Sequence
  Sequence of the HIV-2 R region probe oligo (HIV-2 Pro 3) with reporter and quencher
  misc_feature (1)..(1): Thymine is attached with X wherein X is a reporter molecule
  misc_feature (14)..(14): Guanine is attached with Z wherein Z is a quencher molecule
tccagcactagcag

SEQ ID NO: 43 - DNA, 14 bp, Artificial Sequence
  Sequence of the HIV-2 R region probe oligo (HIV-2 Pro 3) with FAM and BHQ-1
  misc_feature (1)..(1): Thymine is attached with FAM (carboxyfluorescein)
  misc_feature (14)..(14): Guanine is attached with quencher molecule BHQ-1
tccagcactagcag

SEQ ID NO: 44 - DNA, 14 bp, Artificial Sequence
  Sequence of the HIV-2 R region probe oligo (HIV-2 Pro 3) with locked nucleic acids, FAM and BHQ-1
  misc_feature (1)..(1): Thymine is attached with FAM (carboxyfluorescein)
  modified_base (2)..(2): locked nucleic acid cytosine
  modified_base (4)..(4): locked nucleic acid adenine
  modified_base (6)..(6): locked nucleic acid cytosine
  modified_base (8)..(8): locked nucleic acid cytosine
  modified_base (10)..(10): locked nucleic acid adenine
  modified_base (12)..(12): locked nucleic acid cytosine
  misc_feature (14)..(14): Guanine is attached with quencher molecule BHQ-1
tccagcactagcag

SEQ ID NO: 45 - DNA, 16 bp, Artificial Sequence
  Sequence of the HIV-1 R region probe oligo (HIV-1 Pro 2)
  misc_feature (1)..(1): 5-20 nucleotides of T
nggaacccactgctta

SEQ ID NO: 46 - DNA, 15 bp, Artificial Sequence
  Sequence of the HIV-1 R region probe oligo (HIV-1 Pro 2) with reporter and quencher
  misc_feature (1)..(1): Guanine is attached with X wherein X is a reporter molecule
  misc_feature (15)..(15): Adenine is attached with Z wherein Z is a quencher molecule
ggaacccactgctta

SEQ ID NO: 47 - DNA, 15 bp, Artificial Sequence
  Sequence of the HIV-1 R region probe oligo (HIV-1 Pro 3)
agggaacccactgct

SEQ ID NO: 48 - DNA, 15 bp, Artificial Sequence
  Sequence of the HIV-1 R region probe oligo (HIV-1 Pro 3) with reporter and quencher
  misc_feature (1)..(1): Adenine is attached with X wherein X is a reporter molecule
  misc_feature (15)..(15): Thymine is attached with Z wherein Z is a quencher molecule
agggaacccactgct

SEQ ID NO: 49 - DNA, 17 bp, Artificial Sequence
  Sequence of the HIV-2 R region probe oligo (HIV-2 Pro 4)
  misc_feature (1)..(1): 5-20 nucleotides of T
ntccagcactagcaggt

SEQ ID NO: 50 - DNA, 16 bp, Artificial Sequence
  Sequence of the HIV-2 R region probe oligo (HIV-2 Pro 4) with reporter and quencher
  misc_feature (1)..(1): Thymine is attached with X wherein X is a reporter molecule
  misc_feature (16)..(16): Thymine is attached with Z wherein Z is a quencher molecule
tccagcactagcaggt

SEQ ID NO: 51 - DNA, 15 bp, Artificial Sequence
  Sequence of the HIV-2 R region probe oligo (HIV-2 Pro 5)
ctccagcactagcag

SEQ ID NO: 52 - DNA, 15 bp, Artificial Sequence
  Sequence of the HIV-2 R region probe oligo (HIV-2 Pro 5) with reporter and quencher
  misc_feature (1)..(1): Cytosine is attached with X wherein X is a reporter molecule
  misc_feature (15)..(15): Guanine is attached with Z wherein Z is a quencher molecule
ctccagcactagcag

SEQ ID NO: 53 - DNA, 15 bp, Artificial Sequence
  Sequence of the HIV-2 R region probe oligo (HIV-2 Pro-5) with locked nucleic acids
  misc_feature (2)..(2): locked nucleic acid thymine
  misc_feature (5)..(5): locked nucleic acid adenine
  misc_feature (6)..(6): locked nucleic acid guanine
  misc_feature (8)..(8): locked nucleic acid adenine
  misc_feature (11)..(11): locked nucleic acid adenine
  misc_feature (13)..(13): locked nucleic acid cytosine
ctccagcactagcag